European Patent Specification EP 3 060 654 B1, published March 15, 2023. Title: IN VITRO MODEL FOR A TUMOR MICROENVIRONMENT. Applicant: HemoShear, LLC Wamhoff, Brian R Blackman, Brett R Figler, Robert  A Gioeli, Daniel G Simmers, Michael B. The sequence listing filed with the application follows.

SEQUENCE LISTING (74 sequences)

SEQ ID NO: 1 - DNA, 20 bp, Rattus norvegicus
gctgctcttggccgtcacca

SEQ ID NO: 2 - DNA, 20 bp, Rattus norvegicus
tgaagggcaagccccagggt

SEQ ID NO: 3 - DNA, 20 bp, Rattus norvegicus
cctgcgctacctgcccaacc

SEQ ID NO: 4 - DNA, 20 bp, Rattus norvegicus
gggcgcctgtgatgtcctgg

SEQ ID NO: 5 - DNA, 20 bp, Rattus norvegicus
cggcgggattttggcccagt

SEQ ID NO: 6 - DNA, 20 bp, Rattus norvegicus
caggcttgcctgtctccgcc

SEQ ID NO: 7 - DNA, 20 bp, Rattus norvegicus
gctgctgggaactctggcgg

SEQ ID NO: 8 - DNA, 20 bp, Rattus norvegicus
ccggcaccaatgcccgtgta

SEQ ID NO: 9 - DNA, 20 bp, Rattus norvegicus
cgcagcagctatgccaccgt

SEQ ID NO: 10 - DNA, 21 bp, Rattus norvegicus
cttccagctctggccctggtc

SEQ ID NO: 11 - DNA, 24 bp, Rattus norvegicus
agcgttgctccatgggcatatagt

SEQ ID NO: 12 - DNA, 24 bp, Rattus norvegicus
tgtcagggatggtgttggatgaca

SEQ ID NO: 13 - DNA, 24 bp, Rattus norvegicus
tgtcatggttacacccgaagacct

SEQ ID NO: 14 - DNA, 24 bp, Rattus norvegicus
ttgttgttgtttgctcctccaggc

SEQ ID NO: 15 - DNA, 20 bp, Rattus norvegicus
gcgagctctatgggtatatg

SEQ ID NO: 16 - DNA, 20 bp, Rattus norvegicus
agtcctcttcctcagtcctc

SEQ ID NO: 17 - DNA, 24 bp, Rattus norvegicus
atatctccctttttgtggctgcta

SEQ ID NO: 18 - DNA, 22 bp, Rattus norvegicus
tccgactccgtcttctygatga

SEQ ID NO: 19 - DNA, 20 bp, Rattus norvegicus
ggagccatggattgcacatt

SEQ ID NO: 20 - DNA, 21 bp, Rattus norvegicus
aggccagggaagtcactgtct

SEQ ID NO: 21 - DNA, 20 bp, Rattus norvegicus
ctatgtccggacccgcacgc

SEQ ID NO: 22 - DNA, 20 bp, Rattus norvegicus
ctatgtccggacccgcacgc

SEQ ID NO: 23 - DNA, 24 bp, Rattus norvegicus
actctgcaacggagttgtggaaga

SEQ ID NO: 24 - DNA, 24 bp, Rattus norvegicus
tcggatgactccaaccctatcctt

SEQ ID NO: 25 - DNA, 22 bp, Rattus norvegicus
tgtggagccacaggacttacaa

SEQ ID NO: 26 - DNA, 24 bp, Rattus norvegicus
agccaacccacgtgagagaagaaa

SEQ ID NO: 27 - DNA, 24 bp, Rattus norvegicus
atgtggacctgcattccttcccat

SEQ ID NO: 28 - DNA, 24 bp, Rattus norvegicus
ttgcccatgtccttgtaatgtgcg

SEQ ID NO: 29 - DNA, 23 bp, Rattus norvegicus
gaggagtgtggaagaacggattc

SEQ ID NO: 30 - DNA, 21 bp, Rattus norvegicus
aggaactggcggtctgtgtag

SEQ ID NO: 31 - DNA, 21 bp, Rattus norvegicus
tcatcgacacttaccttctgc

SEQ ID NO: 32 - DNA, 22 bp, Rattus norvegicus
agtgtatggcattttggtacga

SEQ ID NO: 33 - DNA, 24 bp, Rattus norvegicus
tctgtggctcggatgttcactact

SEQ ID NO: 34 - DNA, 24 bp, Rattus norvegicus
cggccgatcttgcagaattcatct

SEQ ID NO: 35 - DNA, 22 bp, Rattus norvegicus
ggactatgacaacatccctacc

SEQ ID NO: 36 - DNA, 20 bp, Rattus norvegicus
ccaaccaccttctcctcttt

SEQ ID NO: 37 - DNA, 20 bp, Rattus norvegicus
gcctaagggctttcgttaca

SEQ ID NO: 38 - DNA, 22 bp, Rattus norvegicus
atccacattccaggagcatatc

SEQ ID NO: 39 - DNA, 18 bp, Rattus norvegicus
aggccagcagggagttct

SEQ ID NO: 40 - DNA, 19 bp, Rattus norvegicus
agctcggctccaagttctg

SEQ ID NO: 41 - DNA, 20 bp, Rattus norvegicus
caactcctctccaaggtgct

SEQ ID NO: 42 - DNA, 20 bp, Rattus norvegicus
atctgctcacgcgtgttctt

SEQ ID NO: 43 - DNA, 25 bp, Homo sapiens
ggacctgaatgagaagttctacagc

SEQ ID NO: 44 - DNA, 24 bp, Homo sapiens
agctccaaagaggtccaagacgat

SEQ ID NO: 45 - DNA, 24 bp, Homo sapiens
tcatagccaagaaggtggagcaca

SEQ ID NO: 46 - DNA, 24 bp, Homo sapiens
cccaatgaagaggttcaacgtggt

SEQ ID NO: 47 - DNA, 22 bp, Homo sapiens
gggcacacaggcaagtttacaa

SEQ ID NO: 48 - DNA, 24 bp, Homo sapiens
agagcgtgttgaggttgaggttct

SEQ ID NO: 49 - DNA, 24 bp, Homo sapiens
tgacttgtttggagctgggacaga

SEQ ID NO: 50 - DNA, 22 bp, Homo sapiens
acagcatctgtgtagggcatgt

SEQ ID NO: 51 - DNA, 24 bp, Homo sapiens
acgacactcatcaccaacctgtca

SEQ ID NO: 52 - DNA, 24 bp, Homo sapiens
aggtgaagaagaggaagagctcca

SEQ ID NO: 53 - DNA, 24 bp, Homo sapiens
ctgcattggcatgaggtttgctct

SEQ ID NO: 54 - DNA, 24 bp, Homo sapiens
aaattcaggctccacttacggtgc

SEQ ID NO: 55 - DNA, 24 bp, Homo sapiens
ctgcattggcatgaggtttgctct

SEQ ID NO: 56 - DNA, 24 bp, Homo sapiens
agggttccatctcttgaatccacc

SEQ ID NO: 57 - DNA, 20 bp, Homo sapiens
gatgccaagcttgccttgat

SEQ ID NO: 58 - DNA, 25 bp, Homo sapiens
agggaagctggagataaagactgga

SEQ ID NO: 59 - DNA, 24 bp, Homo sapiens
ggcccatcatgcccaatatggttt

SEQ ID NO: 60 - DNA, 24 bp, Homo sapiens
gcatcagcaattgccatagctttc

SEQ ID NO: 61 - DNA, 23 bp, Homo sapiens
tagcgccaccagaagcgaccaaa

SEQ ID NO: 62 - DNA, 24 bp, Homo sapiens
tcatttgggcctggttcagggata

SEQ ID NO: 63 - DNA, 19 bp, Homo sapiens
ccagccctgtatgaggacc

SEQ ID NO: 64 - DNA, 23 bp, Homo sapiens
ggagctgaccagtattgatgaga

SEQ ID NO: 65 - DNA, 21 bp, Homo sapiens
cacttgcgtgaatgttggatg

SEQ ID NO: 66 - DNA, 20 bp, Homo sapiens
tgggatcactcgtgaaggct

SEQ ID NO: 67 - DNA, 23 bp, Homo sapiens
atatggcaagaaggtgatggtcc

SEQ ID NO: 68 - DNA, 21 bp, Homo sapiens
gggcttgtcctaacaaagctg

SEQ ID NO: 69 - DNA, 24 bp, Canis familiaris
caccatcccccacagcacaacaaa

SEQ ID NO: 70 - DNA, 24 bp, Canis familiaris
gctctggccggaatgcaaatggat

SEQ ID NO: 71 - DNA, 22 bp, Canis familiaris
gagagaatgaaggaaagtcgcc

SEQ ID NO: 72 - DNA, 20 bp, Canis familiaris
gccaccagctccaaatcaga

SEQ ID NO: 73 - DNA, 17 bp, Canis familiaris
tcctcatcctcctcgct

SEQ ID NO: 74 - DNA, 17 bp, Canis familiaris
ttctctgctgggtgtcg